European Patent Specification EP 4 554 563 B1, published February 25, 2026. Title: REVERSED MICELLES FOR DELIVERY OF HYDROPHILIC DRUGS. Applicant: CONSIGLIO NAZIONALE DELLE RICERCHE. Application EP. The sequence listing filed with the application follows.

SEQUENCE LISTING (3 sequences)

SEQ ID NO: 1 - protein, 20 aa, synthetic construct
TFFYGGSRGKRNNFKTEEYG

SEQ ID NO: 2 - protein, 7 aa, synthetic construct
  SITE 3: note = D-Threonine
  CARBOHYD 7: note = O-linked(beta-D-Glucose)
GFTGFLS

SEQ ID NO: 3 - protein, 9 aa, synthetic construct
GGGHKYLRW